European Patent Specification EP 3 443 083 B1, published December 13, 2023. Title: Sequential Loadings of Multiple Delivery Vectors Using a Single Selectable Markers. Applicant: Perkins, Edward. Application Filed herewith. The sequence listing filed with the application follows.

SEQUENCE LISTING (14 sequences)

SEQ ID NO: 1 - DNA, 24 bp, Artificial Sequence
  ligation junction
accgagctgcaagaactcttcctc

SEQ ID NO: 2 - DNA, 18 bp, Artificial Sequence
  ligation junction
ctcgccgcagccgtgtaa

SEQ ID NO: 3 - DNA, 22 bp, Artificial Sequence
  ligation junction
gcgctaatgctctgttacaggt

SEQ ID NO: 4 - DNA, 20 bp, Artificial Sequence
  ligation junction
ggaaagctgccagtgccttg

SEQ ID NO: 5 - DNA, 53 bp, Artificial Sequence
  lox cassette
agccgtgtaaccgagcatagtgaagcctgcttttttatactaacttgagcgaa

SEQ ID NO: 6 - DNA, 43 bp, Artificial Sequence
  lox cassette
ctgtttccttcagcctgcatggccttgactagagggtcgacgg

SEQ ID NO: 7 - DNA, 34 bp, Artificial Sequence
  loxP
ataacttcgtataatgtatgctatacgaagttat

SEQ ID NO: 8 - protein, 11 aa, Artificial Sequence
  loxP
ITSYNVCYTKL

SEQ ID NO: 9 - DNA, 34 bp, Artificial Sequence
  lox5171
ataacttcgtataatgtgtactatacgaagttat

SEQ ID NO: 10 - protein, 11 aa, Artificial Sequence
  lox5171
ITSYNVYYTKL

SEQ ID NO: 11 - DNA, 34 bp, Artificial Sequence
  lox2272
ataacttcgtataaagtatcctatacgaagttat

SEQ ID NO: 12 - protein, 11 aa, Artificial Sequence
  lox2272
ITSYKVSYTKL

SEQ ID NO: 13 - DNA, 34 bp, Artificial Sequence
  loxM2
ataacttcgtataagaaaccatatacgaagttat

SEQ ID NO: 14 - protein, 11 aa, Artificial Sequence
  loxM2
ITSYKKPYTKL